European Patent Application EP 4 261 286 A1, published October 18, 2023. Title: Shewanella atlantica-Drived Protein Expressing Microorganism and Method of L-Amino Acid Production Using the Same. Applicant: CJ CheilJedang Corporation. The sequence listing filed with the application follows.

SEQUENCE LISTING (10 sequences)

SEQ ID NO: 1 - protein, 202 aa, Artificial Sequence
  Membrane protein derived from Shewanella atlantica (Sat)
MQAFIQGVGIGGSLIMAVGAQNAFVLKQGLKRSHSLPIAGLCSLIDALMITAGVAGLGHLILAFPLIKDIASIGGAIFLLVYGAKALRSSFNEQTISQGATKGTETLKAAVLTTLGISLLNPHLYLDTVVLLGSISAQFEGVDRPLFGAGAVLASFVWFFSLSFGARYLSPLFQNPKAWSYLDRFICMTMWTIAAVLLWPYL

SEQ ID NO: 2 - DNA, 609 bp, Artificial Sequence
  Sat coding nucleotide sequence
atgcaggcatttattcagggtgtaggaattggcggaagccttattatggcggtgggcgcacaaaatgcgtttgtattaaagcaggggctgaagcgttcgcactctttacccattgccggactgtgttcattgatcgatgccttaatgataacggctggtgtggcaggcctgggtcatttgattttggcctttccattgattaaggatattgccagtattggtggggcgatcttcttgctggtttatggtgcaaaggctttaaggtcttcgtttaatgagcaaaccatatctcaaggtgcgacgaaagggactgaaacccttaaagctgcggtgttgacaactttgggtattagtttgctcaacccgcatctgtatctggacacggttgtcttgcttggtagcatcagtgctcagtttgaaggtgttgaccgtcctctgtttggcgcaggtgccgtactggcatcgtttgtgtggttttttagtttaagttttggtgcgagatacttaagtccattatttcaaaaccctaaagcctggagctatttagacaggtttatctgcatgactatgtggaccattgcggcggtcttgttatggccttacttgtaa

SEQ ID NO: 3 - DNA, 35 bp, Artificial Sequence
  Sat-F_primer
tagaggagacacaacatgcaggcatttattcaggg

SEQ ID NO: 4 - DNA, 36 bp, Artificial Sequence
  Sat-R_primer
tagatgtcgggcccattacaagtaaggccataacaa

SEQ ID NO: 5 - DNA, 35 bp, Artificial Sequence
  PgapA-F_primer
aatgagttcctcgagaaacgaccgagcctattggg

SEQ ID NO: 6 - DNA, 35 bp, Artificial Sequence
  PgapA-R_primer
taaatgcctgcatgttgtgtctcctctaaagattg

SEQ ID NO: 7 - DNA, 20 bp, Artificial Sequence
  pDZTn-1_primer
acgacgctggtatttctccc

SEQ ID NO: 8 - DNA, 20 bp, Artificial Sequence
  pDZTn-2_primer
tgattgtcgatatgaccggg

SEQ ID NO: 9 - DNA, 20 bp, Artificial Sequence
  Tn-1_primer
taaggcaccgcagaatgtag

SEQ ID NO: 10 - DNA, 20 bp, Artificial Sequence
  Tn-2_primer
taggactcaccatcaccggc